European Patent Application EP 4 316 512 A2, published February 7, 2024. Title: INTRATHECAL ADMINISTRATION OF ADENO-ASSOCIATED-VIRAL VECTORS FOR GENE THERAPY. Applicant: The Trustees of The University of Pennsylvania. Application EP. The sequence listing filed with the application follows.

SEQUENCE LISTING (15 sequences)

SEQ ID NO: 1 - DNA, 6694 bp, synthetic construct
  misc_feature 1..6694: note = pAAV.CB7.CI.201IA.rBG
  regulatory 60..186: regulatory_class = polyA_signal_sequence
  misc_feature 275..404: note = 3' ITR (complement)
  rep_origin 581..1036
  misc_feature 3226..3355: note = 5' ITR
  misc_feature 3423..3804: note = misc - CMV IE promoter
  regulatory 3807..4088: regulatory_class = promoter
  regulatory 4061..4064: regulatory_class = TATA_box
  misc_feature 4183..5155: note = Intron
  source 1..6694: mol_type = other DNA
  CDS 5161..6690: note = 201IA; protein_id = 2; translation = MEFGLSWVFLVALLKGVQCEVQLLESGPGLVKPSETLSLTCAVSGLSISSDFSWAWIRQTPGKALEYVGYIRGNTGDTYYNPSLKSRLTISKDTSKNQIYLNLSSVTAGDAAVYYCARDRVCDDDYGYYYTEVCFGLDSWGQGIVVTVSSGGGGSGGGGSGGGGSAELVMTQSPLSLSVAPGQTASISCRSSQSLDYANGNTYLSWFHQRPGQPPRRLIYQISNRDSGVPDRFSGSGAGTEFTLRISRMESDDVGIYYCGQGTTFPRTFGQGTKVEIKTCGGGSKPPTCPPCTSPELLGGPSVFLFPPKPKDTLMISRTPEVTCVVVDVSQEDPDVKFNWYVNGAEVHHAQTKPRETQYNSTYRVVSVLTVTHQDWLNGKEYTCKVSNKALPAPIQKTISKDKGQPREPQVYTLPPSREELTKNQVSLTCLVKGFYPSDIVVEWESSGQPENTYKTTPPVLDSDGSYFLYSKLTVDKSRWQQGNVFSCSVMHEALHNHYTQKSLSLSPGK
gtacctctagagtcgacccgggcggcctcgaggacggggtgaactacgcctgaggatccgatctttttccctctgccaaaaattatggggacatcatgaagccccttgagcatctgacttctggctaataaaggaaatttattttcattgcaatagtgtgttggaattttttgtgtctctcactcggaagcaattcgttgatctgaatttcgaccacccataatacccattaccctggtagataagtagcatggcgggttaatcattaactacaaggaacccctagtgatggagttggccactccctctctgcgcgctcgctcgctcactgaggccgggcgaccaaaggtcgcccgacgcccgggctttgcccgggcggcctcagtgagcgagcgagcgcgcagccttaattaacctaattcactggccgtcgttttacaacgtcgtgactgggaaaaccctggcgttacccaacttaatcgccttgcagcacatccccctttcgccagctggcgtaatagcgaagaggcccgcaccgatcgcccttcccaacagttgcgcagcctgaatggcgaatgggacgcgccctgtagcggcgcattaagcgcggcgggtgtggtggttacgcgcagcgtgaccgctacacttgccagcgccctagcgcccgctcctttcgctttcttcccttcctttctcgccacgttcgccggctttccccgtcaagctctaaatcgggggctccctttagggttccgatttagtgctttacggcacctcgaccccaaaaaacttgattagggtgatggttcacgtagtgggccatcgccctgatagacggtttttcgccctttgacgttggagtccacgttctttaatagtggactcttgttccaaactggaacaacactcaaccctatctcggtctattcttttgatttataagggattttgccgatttcggcctattggttaaaaaatgagctgatttaacaaaaatttaacgcgaattttaacaaaatattaacgcttacaatttaggtggcacttttcggggaaatgtgcgcggaacccctatttgtttatttttctaaatacattcaaatatgtatccgctcatgagacaataaccctgataaatgcttcaataatattgaaaaaggaagagtatgagtattcaacatttccgtgtcgcccttattcccttttttgcggcattttgccttcctgtttttgctcacccagaaacgctggtgaaagtaaaagatgctgaagatcagttgggtgcacgagtgggttacatcgaactggatctcaacagcggtaagatccttgagagttttcgccccgaagaacgttttccaatgatgagcacttttaaagttctgctatgtggcgcggtattatcccgtattgacgccgggcaagagcaactcggtcgccgcatacactattctcagaatgacttggttgagtactcaccagtcacagaaaagcatcttacggatggcatgacagtaagagaattatgcagtgctgccataaccatgagtgataacactgcggccaacttacttctgacaacgatcggaggaccgaaggagctaaccgcttttttgcacaacatgggggatcatgtaactcgccttgatcgttgggaaccggagctgaatgaagccataccaaacgacgagcgtgacaccacgatgcctgtagcaatggcaacaacgttgcgcaaactattaactggcgaactacttactctagcttcccggcaacaattaatagactggatggaggcggataaagttgcaggaccacttctgcgctcggcccttccggctggctggtttattgctgataaatctggagccggtgagcgtgggtctcgcggtatcattgcagcactggggccagatggtaagccctcccgtatcgtagttatctacacgacggggagtcaggcaactatggatgaacgaaatagacagatcgctgagataggtgcctcactgattaagcattggtaactgtcagaccaagtttactcatatatactttagattgatttaaaacttcatttttaatttaaaaggatctaggtgaagatcctttttgataatctcatgaccaaaatcccttaacgtgagttttcgttccactgagcgtcagaccccgtagaaaagatcaaaggatcttcttgagatcctttttttctgcgcgtaatctgctgcttgcaaacaaaaaaaccaccgctaccagcggtggtttgtttgccggatcaagagctaccaactctttttccgaaggtaactggcttcagcagagcgcagataccaaatactgttcttctagtgtagccgtagttaggccaccacttcaagaactctgtagcaccgcctacatacctcgctctgctaatcctgttaccagtggctgctgccagtggcgataagtcgtgtcttaccgggttggactcaagacgatagttaccggataaggcgcagcggtcgggctgaacggggggttcgtgcacacagcccagcttggagcgaacgacctacaccgaactgagatacctacagcgtgagctatgagaaagcgccacgcttcccgaagggagaaaggcggacaggtatccggtaagcggcagggtcggaacaggagagcgcacgagggagcttccagggggaaacgcctggtatctttatagtcctgtcgggtttcgccacctctgacttgagcgtcgatttttgtgatgctcgtcaggggggcggagcctatggaaaaacgccagcaacgcggcctttttacggttcctggccttttgctggccttttgctcacatgttctttcctgcgttatcccctgattctgtggataaccgtattaccgcctttgagtgagctgataccgctcgccgcagccgaacgaccgagcgcagcgagtcagtgagcgaggaagcggaagagcgcccaatacgcaaaccgcctctccccgcgcgttggccgattcattaatgcagctggcacgacaggtttcccgactggaaagcgggcagtgagcgcaacgcaattaatgtgagttagctcactcattaggcaccccaggctttacactttatgcttccggctcgtatgttgtgtggaattgtgagcggataacaatttcacacaggaaacagctatgaccatgattacgccagatttaattaaggccttaattaggctgcgcgctcgctcgctcactgaggccgcccgggcaaagcccgggcgtcgggcgacctttggtcgcccggcctcagtgagcgagcgagcgcgcagagagggagtggccaactccatcactaggggttccttgtagttaatgattaacccgccatgctacttatctaccagggtaatggggatcctctagaactatagctagtcgacattgattattgactagttattaatagtaatcaattacggggtcattagttcatagcccatatatggagttccgcgttacataacttacggtaaatggcccgcctggctgaccgcccaacgacccccgcccattgacgtcaataatgacgtatgttcccatagtaacgccaatagggactttccattgacgtcaatgggtggactatttacggtaaactgcccacttggcagtacatcaagtgtatcatatgccaagtacgccccctattgacgtcaatgacggtaaatggcccgcctggcattatgcccagtacatgaccttatgggactttcctacttggcagtacatctacgtattagtcatcgctattaccatggtcgaggtgagccccacgttctgcttcactctccccatctcccccccctccccacccccaattttgtatttatttattttttaattattttgtgcagcgatgggggcggggggggggggggggcgcgcgccaggcggggcggggcggggcgaggggcggggcggggcgaggcggagaggtgcggcggcagccaatcagagcggcgcgctccgaaagtttccttttatggcgaggcggcggcggcggcggccctataaaaagcgaagcgcgcggcgggcggggagtcgctgcgacgctgccttcgccccgtgccccgctccgccgccgcctcgcgccgcccgccccggctctgactgaccgcgttactcccacaggtgagcgggcgggacggcccttctcctccgggctgtaattagcgcttggtttaatgacggcttgtttcttttctgtggctgcgtgaaagccttgaggggctccgggagggccctttgtgcggggggagcggctcggggggtgcgtgcgtgtgtgtgtgcgtggggagcgccgcgtgcggctccgcgctgcccggcggctgtgagcgctgcgggcgcggcgcggggctttgtgcgctccgcagtgtgcgcgaggggagcgcggccgggggcggtgccccgcggtgcggggggggctgcgaggggaacaaaggctgcgtgcggggtgtgtgcgtgggggggtgagcagggggtgtgggcgcgtcggtcgggctgcaaccccccctgcacccccctccccgagttgctgagcacggcccggcttcgggtgcggggctccgtacggggcgtggcgcggggctcgccgtgccgggcggggggtggcggcaggtgggggtgccgggcggggcggggccgcctcgggccggggagggctcgggggaggggcgcggcggcccccggagcgccggcggctgtcgaggcgcggcgagccgcagccattgccttttatggtaatcgtgcgagagggcgcagggacttcctttgtcccaaatctgtgcggagccgaaatctgggaggcgccgccgcaccccctctagcgggcgcggggcgaagcggtgcggcgccggcaggaaggaaatgggcggggagggccttcgtgcgtcgccgcgccgccgtccccttctccctctccagcctcggggctgtccgcggggggacggctgccttcgggggggacggggcagggcggggttcggcttctggcgtgtgaccggcggctctagagcctctgctaaccatgttcatgccttcttctttttcctacagctcctgggcaacgtgctggttattgtgctgtctcatcattttggcaaagaattcatggagttcgggctgagctgggtctttctggtggccctgctgaagggagtccagtgcgaggtgcagctgctggaatccggacctggcctggtgaaaccatctgagacactgagtctgacttgtgctgtctccggcctgtctatcagctccgatttctcctgggcatggattaggcagacccccggcaaggccctggaatatgtggggtacatccgcgggaacaccggagatacatactataatcctagtctgaagtcaaggctgactatctcaaaggacaccagcaaaaaccaaatctacctgaatctgtctagtgtcaccgctggcgatgccgccgtgtactattgcgcaagggaccgggtgtgcgacgatgactacggatactattacaccgaggtgtgcttcggcctggattcttgggggcagggaatcgtggtcacagtgtcaagcggcggaggaggcagcggaggaggagggtccggaggcgggggatctgcagaactggtcatgacacagtccccactgagcctgtccgtcgctccaggacagactgcatctattagttgtcgatcctctcagtccctggactatgctaacggcaatacctacctgtcttggtttcaccagcgaccaggacagccacctcggagactgatctatcagatttccaacagagattctggagtgcccgacaggttctcaggcagcggagcaggaactgagtttaccctgcgaatcagtcggatggaatcagatgacgtggggatctactactgcggacaggggaccacattcccacggacatttggacagggcactaaggtggagatcaaaacctgtggaggaggaagcaagccaccaacctgccctccatgtacatctcccgaactgctgggcgggcctagcgtgttcctgtttccccctaagcctaaagatacactgatgattagtagaaccccagaggtcacatgcgtggtcgtggacgtgtcccaggaagatcctgacgtgaagttcaactggtacgtgaatggcgccgaggtgcaccatgctcagactaaaccacgcgaaacccagtataatagtacataccgagtcgtgtcagtcctgacagtgactcaccaggattggctgaacggcaaggagtatacctgcaaggtgtctaacaaggccctgcccgcccctatccagaaaacaattagcaaggacaaagggcagccacgggaaccccaggtgtacactctgccaccctcaagagaggaactgactaagaaccaggtcagcctgacctgtctggtgaaaggcttctaccccagcgatatcgtcgtggagtgggaaagttcaggccagcctgagaatacttacaagactacccctccagtgctggatagcgacgggtcctatttcctgtacagcaagctgacagtggacaaatcccgctggcagcagggaaacgtcttttcctgttctgtgatgcatgaggccctgcacaatcattacacccagaagagtctgtcactgagccccggcaaatgag

SEQ ID NO: 2 - protein, 510 aa, synthetic construct
  REGION 1..510: note = Synthetic Construct
MEFGLSWVFLVALLKGVQCEVQLLESGPGLVKPSETLSLTCAVSGLSISSDFSWAWIRQTPGKALEYVGYIRGNTGDTYYNPSLKSRLTISKDTSKNQIYLNLSSVTAGDAAVYYCARDRVCDDDYGYYYTEVCFGLDSWGQGIVVTVSSGGGGSGGGGSGGGGSAELVMTQSPLSLSVAPGQTASISCRSSQSLDYANGNTYLSWFHQRPGQPPRRLIYQISNRDSGVPDRFSGSGAGTEFTLRISRMESDDVGIYYCGQGTTFPRTFGQGTKVEIKTCGGGSKPPTCPPCTSPELLGGPSVFLFPPKPKDTLMISRTPEVTCVVVDVSQEDPDVKFNWYVNGAEVHHAQTKPRETQYNSTYRVVSVLTVTHQDWLNGKEYTCKVSNKALPAPIQKTISKDKGQPREPQVYTLPPSREELTKNQVSLTCLVKGFYPSDIVVEWESSGQPENTYKTTPPVLDSDGSYFLYSKLTVDKSRWQQGNVFSCSVMHEALHNHYTQKSLSLSPGK

SEQ ID NO: 3 - DNA, 6694 bp, synthetic construct
  misc_feature 1..6694: note = Plasmid encoding 201IA(I253A)mutant
  misc_feature 1..130: note = misc - 5' ITR
  misc_feature 198..579: note = CMV IE promoter
  regulatory 582..863: note = promoter - CB promoter; regulatory_class = promoter
  regulatory 836..839: regulatory_class = TATA_box
  misc_feature 958..1930: note = Intron - chicken beta-actin intron
  regulatory 3529..3655: note = polyA_signal - rabbit globin polyA; regulatory_class = polyA_signal_sequence
  misc_feature 3744..3873: note = 3' ITR (complement)
  rep_origin 4050..4505
  misc_feature 4636..5493: note = AP(R) marker
  rep_origin 5667..6255
  source 1..6694: mol_type = other DNA
  CDS 1936..3465: note = 201IA; protein_id = 4; translation = MEFGLSWVFLVALLKGVQCEVQLLESGPGLVKPSETLSLTCAVSGLSISSDFSWAWIRQTPGKALEYVGYIRGNTGDTYYNPSLKSRLTISKDTSKNQIYLNLSSVTAGDAAVYYCARDRVCDDDYGYYYTEVCFGLDSWGQGIVVTVSSGGGGSGGGGSGGGGSAELVMTQSPLSLSVAPGQTASISCRSSQSLDYANGNTYLSWFHQRPGQPPRRLIYQISNRDSGVPDRFSGSGAGTEFTLRISRMESDDVGIYYCGQGTTFPRTFGQGTKVEIKTCGGGSKPPTCPPCTSPELLGGPSVFLFPPKPKDTLMASRTPEVTCVVVDVSQEDPDVKFNWYVNGAEVHHAQTKPRETQYNSTYRVVSVLTVTHQDWLNGKEYTCKVSNKALPAPIQKTISKDKGQPREPQVYTLPPSREELTKNQVSLTCLVKGFYPSDIVVEWESSGQPENTYKTTPPVLDSDGSYFLYSKLTVDKSRWQQGNVFSCSVMHEALHNHYTQKSLSLSPGK
ctgcgcgctcgctcgctcactgaggccgcccgggcaaagcccgggcgtcgggcgacctttggtcgcccggcctcagtgagcgagcgagcgcgcagagagggagtggccaactccatcactaggggttccttgtagttaatgattaacccgccatgctacttatctaccagggtaatggggatcctctagaactatagctagtcgacattgattattgactagttattaatagtaatcaattacggggtcattagttcatagcccatatatggagttccgcgttacataacttacggtaaatggcccgcctggctgaccgcccaacgacccccgcccattgacgtcaataatgacgtatgttcccatagtaacgccaatagggactttccattgacgtcaatgggtggactatttacggtaaactgcccacttggcagtacatcaagtgtatcatatgccaagtacgccccctattgacgtcaatgacggtaaatggcccgcctggcattatgcccagtacatgaccttatgggactttcctacttggcagtacatctacgtattagtcatcgctattaccatggtcgaggtgagccccacgttctgcttcactctccccatctcccccccctccccacccccaattttgtatttatttattttttaattattttgtgcagcgatgggggcggggggggggggggggcgcgcgccaggcggggcggggcggggcgaggggcggggcggggcgaggcggagaggtgcggcggcagccaatcagagcggcgcgctccgaaagtttccttttatggcgaggcggcggcggcggcggccctataaaaagcgaagcgcgcggcgggcggggagtcgctgcgacgctgccttcgccccgtgccccgctccgccgccgcctcgcgccgcccgccccggctctgactgaccgcgttactcccacaggtgagcgggcgggacggcccttctcctccgggctgtaattagcgcttggtttaatgacggcttgtttcttttctgtggctgcgtgaaagccttgaggggctccgggagggccctttgtgcggggggagcggctcggggggtgcgtgcgtgtgtgtgtgcgtggggagcgccgcgtgcggctccgcgctgcccggcggctgtgagcgctgcgggcgcggcgcggggctttgtgcgctccgcagtgtgcgcgaggggagcgcggccgggggcggtgccccgcggtgcggggggggctgcgaggggaacaaaggctgcgtgcggggtgtgtgcgtgggggggtgagcagggggtgtgggcgcgtcggtcgggctgcaaccccccctgcacccccctccccgagttgctgagcacggcccggcttcgggtgcggggctccgtacggggcgtggcgcggggctcgccgtgccgggcggggggtggcggcaggtgggggtgccgggcggggcggggccgcctcgggccggggagggctcgggggaggggcgcggcggcccccggagcgccggcggctgtcgaggcgcggcgagccgcagccattgccttttatggtaatcgtgcgagagggcgcagggacttcctttgtcccaaatctgtgcggagccgaaatctgggaggcgccgccgcaccccctctagcgggcgcggggcgaagcggtgcggcgccggcaggaaggaaatgggcggggagggccttcgtgcgtcgccgcgccgccgtccccttctccctctccagcctcggggctgtccgcggggggacggctgccttcgggggggacggggcagggcggggttcggcttctggcgtgtgaccggcggctctagagcctctgctaaccatgttcatgccttcttctttttcctacagctcctgggcaacgtgctggttattgtgctgtctcatcattttggcaaagaattcatggagttcgggctgagctgggtctttctggtggccctgctgaagggagtccagtgcgaggtgcagctgctggaatccggacctggcctggtgaaaccatctgagacactgagtctgacttgtgctgtctccggcctgtctatcagctccgatttctcctgggcatggattaggcagacccccggcaaggccctggaatatgtggggtacatccgcgggaacaccggagatacatactataatcctagtctgaagtcaaggctgactatctcaaaggacaccagcaaaaaccaaatctacctgaatctgtctagtgtcaccgctggcgatgccgccgtgtactattgcgcaagggaccgggtgtgcgacgatgactacggatactattacaccgaggtgtgcttcggcctggattcttgggggcagggaatcgtggtcacagtgtcaagcggcggaggaggcagcggaggaggagggtccggaggcgggggatctgcagaactggtcatgacacagtccccactgagcctgtccgtcgctccaggacagactgcatctattagttgtcgatcctctcagtccctggactatgctaacggcaatacctacctgtcttggtttcaccagcgaccaggacagccacctcggagactgatctatcagatttccaacagagattctggagtgcccgacaggttctcaggcagcggagcaggaactgagtttaccctgcgaatcagtcggatggaatcagatgacgtggggatctactactgcggacaggggaccacattcccacggacatttggacagggcactaaggtggagatcaaaacctgtggaggaggaagcaagccaccaacctgccctccatgtacatctcccgaactgctgggcgggcctagcgtgttcctgtttccccctaagcctaaagatacactgatggccagtagaaccccagaggtcacatgcgtggtcgtggacgtgtcccaggaagatcctgacgtgaagttcaactggtacgtgaatggcgccgaggtgcaccatgctcagactaaaccacgcgaaacccagtataatagtacataccgagtcgtgtcagtcctgacagtgactcaccaggattggctgaacggcaaggagtatacctgcaaggtgtctaacaaggccctgcccgcccctatccagaaaacaattagcaaggacaaagggcagccacgggaaccccaggtgtacactctgccaccctcaagagaggaactgactaagaaccaggtcagcctgacctgtctggtgaaaggcttctaccccagcgatatcgtcgtggagtgggaaagttcaggccagcctgagaatacttacaagactacccctccagtgctggatagcgacgggtcctatttcctgtacagcaagctgacagtggacaaatcccgctggcagcagggaaacgtcttttcctgttctgtgatgcatgaggccctgcacaatcattacacccagaagagtctgtcactgagccccggcaaatgaggtacctctagagtcgacccgggcggcctcgaggacggggtgaactacgcctgaggatccgatctttttccctctgccaaaaattatggggacatcatgaagccccttgagcatctgacttctggctaataaaggaaatttattttcattgcaatagtgtgttggaattttttgtgtctctcactcggaagcaattcgttgatctgaatttcgaccacccataatacccattaccctggtagataagtagcatggcgggttaatcattaactacaaggaacccctagtgatggagttggccactccctctctgcgcgctcgctcgctcactgaggccgggcgaccaaaggtcgcccgacgcccgggctttgcccgggcggcctcagtgagcgagcgagcgcgcagccttaattaacctaattcactggccgtcgttttacaacgtcgtgactgggaaaaccctggcgttacccaacttaatcgccttgcagcacatccccctttcgccagctggcgtaatagcgaagaggcccgcaccgatcgcccttcccaacagttgcgcagcctgaatggcgaatgggacgcgccctgtagcggcgcattaagcgcggcgggtgtggtggttacgcgcagcgtgaccgctacacttgccagcgccctagcgcccgctcctttcgctttcttcccttcctttctcgccacgttcgccggctttccccgtcaagctctaaatcgggggctccctttagggttccgatttagtgctttacggcacctcgaccccaaaaaacttgattagggtgatggttcacgtagtgggccatcgccctgatagacggtttttcgccctttgacgttggagtccacgttctttaatagtggactcttgttccaaactggaacaacactcaaccctatctcggtctattcttttgatttataagggattttgccgatttcggcctattggttaaaaaatgagctgatttaacaaaaatttaacgcgaattttaacaaaatattaacgcttacaatttaggtggcacttttcggggaaatgtgcgcggaacccctatttgtttatttttctaaatacattcaaatatgtatccgctcatgagacaataaccctgataaatgcttcaataatattgaaaaaggaagagtatgagtattcaacatttccgtgtcgcccttattcccttttttgcggcattttgccttcctgtttttgctcacccagaaacgctggtgaaagtaaaagatgctgaagatcagttgggtgcacgagtgggttacatcgaactggatctcaacagcggtaagatccttgagagttttcgccccgaagaacgttttccaatgatgagcacttttaaagttctgctatgtggcgcggtattatcccgtattgacgccgggcaagagcaactcggtcgccgcatacactattctcagaatgacttggttgagtactcaccagtcacagaaaagcatcttacggatggcatgacagtaagagaattatgcagtgctgccataaccatgagtgataacactgcggccaacttacttctgacaacgatcggaggaccgaaggagctaaccgcttttttgcacaacatgggggatcatgtaactcgccttgatcgttgggaaccggagctgaatgaagccataccaaacgacgagcgtgacaccacgatgcctgtagcaatggcaacaacgttgcgcaaactattaactggcgaactacttactctagcttcccggcaacaattaatagactggatggaggcggataaagttgcaggaccacttctgcgctcggcccttccggctggctggtttattgctgataaatctggagccggtgagcgtgggtctcgcggtatcattgcagcactggggccagatggtaagccctcccgtatcgtagttatctacacgacggggagtcaggcaactatggatgaacgaaatagacagatcgctgagataggtgcctcactgattaagcattggtaactgtcagaccaagtttactcatatatactttagattgatttaaaacttcatttttaatttaaaaggatctaggtgaagatcctttttgataatctcatgaccaaaatcccttaacgtgagttttcgttccactgagcgtcagaccccgtagaaaagatcaaaggatcttcttgagatcctttttttctgcgcgtaatctgctgcttgcaaacaaaaaaaccaccgctaccagcggtggtttgtttgccggatcaagagctaccaactctttttccgaaggtaactggcttcagcagagcgcagataccaaatactgttcttctagtgtagccgtagttaggccaccacttcaagaactctgtagcaccgcctacatacctcgctctgctaatcctgttaccagtggctgctgccagtggcgataagtcgtgtcttaccgggttggactcaagacgatagttaccggataaggcgcagcggtcgggctgaacggggggttcgtgcacacagcccagcttggagcgaacgacctacaccgaactgagatacctacagcgtgagctatgagaaagcgccacgcttcccgaagggagaaaggcggacaggtatccggtaagcggcagggtcggaacaggagagcgcacgagggagcttccagggggaaacgcctggtatctttatagtcctgtcgggtttcgccacctctgacttgagcgtcgatttttgtgatgctcgtcaggggggcggagcctatggaaaaacgccagcaacgcggcctttttacggttcctggccttttgctggccttttgctcacatgttctttcctgcgttatcccctgattctgtggataaccgtattaccgcctttgagtgagctgataccgctcgccgcagccgaacgaccgagcgcagcgagtcagtgagcgaggaagcggaagagcgcccaatacgcaaaccgcctctccccgcgcgttggccgattcattaatgcagctggcacgacaggtttcccgactggaaagcgggcagtgagcgcaacgcaattaatgtgagttagctcactcattaggcaccccaggctttacactttatgcttccggctcgtatgttgtgtggaattgtgagcggataacaatttcacacaggaaacagctatgaccatgattacgccagatttaattaaggccttaattagg

SEQ ID NO: 4 - protein, 510 aa, synthetic construct
  REGION 1..510: note = Synthetic Construct
MEFGLSWVFLVALLKGVQCEVQLLESGPGLVKPSETLSLTCAVSGLSISSDFSWAWIRQTPGKALEYVGYIRGNTGDTYYNPSLKSRLTISKDTSKNQIYLNLSSVTAGDAAVYYCARDRVCDDDYGYYYTEVCFGLDSWGQGIVVTVSSGGGGSGGGGSGGGGSAELVMTQSPLSLSVAPGQTASISCRSSQSLDYANGNTYLSWFHQRPGQPPRRLIYQISNRDSGVPDRFSGSGAGTEFTLRISRMESDDVGIYYCGQGTTFPRTFGQGTKVEIKTCGGGSKPPTCPPCTSPELLGGPSVFLFPPKPKDTLMASRTPEVTCVVVDVSQEDPDVKFNWYVNGAEVHHAQTKPRETQYNSTYRVVSVLTVTHQDWLNGKEYTCKVSNKALPAPIQKTISKDKGQPREPQVYTLPPSREELTKNQVSLTCLVKGFYPSDIVVEWESSGQPENTYKTTPPVLDSDGSYFLYSKLTVDKSRWQQGNVFSCSVMHEALHNHYTQKSLSLSPGK

SEQ ID NO: 5 - DNA, 6694 bp, synthetic construct
  misc_feature 1..6694: note = engineered plasmid containining 201IA(H435) mutant
  misc_feature 275..404: note = 3' ITR (complement)
  rep_origin 2198..2786
  misc_feature 3226..3355
  misc_feature 3423..3804: note = CMV IE promoter
  regulatory 3807..4088: note = promoter - CB promoter; regulatory_class = promoter
  regulatory 4061..4064: note = TATA_signal - rabbit globin polyA; regulatory_class = TATA_box
  misc_feature 4183..5155: note = Intron - chicken beta-actin intron
  source 1..6694: mol_type = other DNA
  CDS 5161..6690: note = 201IA; protein_id = 6; translation = MEFGLSWVFLVALLKGVQCEVQLLESGPGLVKPSETLSLTCAVSGLSISSDFSWAWIRQTPGKALEYVGYIRGNTGDTYYNPSLKSRLTISKDTSKNQIYLNLSSVTAGDAAVYYCARDRVCDDDYGYYYTEVCFGLDSWGQGIVVTVSSGGGGSGGGGSGGGGSAELVMTQSPLSLSVAPGQTASISCRSSQSLDYANGNTYLSWFHQRPGQPPRRLIYQISNRDSGVPDRFSGSGAGTEFTLRISRMESDDVGIYYCGQGTTFPRTFGQGTKVEIKTCGGGSKPPTCPPCTSPELLGGPSVFLFPPKPKDTLMISRTPEVTCVVVDVSQEDPDVKFNWYVNGAEVHHAQTKPRETQYNSTYRVVSVLTVTHQDWLNGKEYTCKVSNKALPAPIQKTISKDKGQPREPQVYTLPPSREELTKNQVSLTCLVKGFYPSDIVVEWESSGQPENTYKTTPPVLDSDGSYFLYSKLTVDKSRWQQGNVFSCSVMHEALHNAYTQKSLSLSPGK
gtacctctagagtcgacccgggcggcctcgaggacggggtgaactacgcctgaggatccgatctttttccctctgccaaaaattatggggacatcatgaagccccttgagcatctgacttctggctaataaaggaaatttattttcattgcaatagtgtgttggaattttttgtgtctctcactcggaagcaattcgttgatctgaatttcgaccacccataatacccattaccctggtagataagtagcatggcgggttaatcattaactacaaggaacccctagtgatggagttggccactccctctctgcgcgctcgctcgctcactgaggccgggcgaccaaaggtcgcccgacgcccgggctttgcccgggcggcctcagtgagcgagcgagcgcgcagccttaattaacctaattcactggccgtcgttttacaacgtcgtgactgggaaaaccctggcgttacccaacttaatcgccttgcagcacatccccctttcgccagctggcgtaatagcgaagaggcccgcaccgatcgcccttcccaacagttgcgcagcctgaatggcgaatgggacgcgccctgtagcggcgcattaagcgcggcgggtgtggtggttacgcgcagcgtgaccgctacacttgccagcgccctagcgcccgctcctttcgctttcttcccttcctttctcgccacgttcgccggctttccccgtcaagctctaaatcgggggctccctttagggttccgatttagtgctttacggcacctcgaccccaaaaaacttgattagggtgatggttcacgtagtgggccatcgccctgatagacggtttttcgccctttgacgttggagtccacgttctttaatagtggactcttgttccaaactggaacaacactcaaccctatctcggtctattcttttgatttataagggattttgccgatttcggcctattggttaaaaaatgagctgatttaacaaaaatttaacgcgaattttaacaaaatattaacgcttacaatttaggtggcacttttcggggaaatgtgcgcggaacccctatttgtttatttttctaaatacattcaaatatgtatccgctcatgagacaataaccctgataaatgcttcaataatattgaaaaaggaagagtatgagtattcaacatttccgtgtcgcccttattcccttttttgcggcattttgccttcctgtttttgctcacccagaaacgctggtgaaagtaaaagatgctgaagatcagttgggtgcacgagtgggttacatcgaactggatctcaacagcggtaagatccttgagagttttcgccccgaagaacgttttccaatgatgagcacttttaaagttctgctatgtggcgcggtattatcccgtattgacgccgggcaagagcaactcggtcgccgcatacactattctcagaatgacttggttgagtactcaccagtcacagaaaagcatcttacggatggcatgacagtaagagaattatgcagtgctgccataaccatgagtgataacactgcggccaacttacttctgacaacgatcggaggaccgaaggagctaaccgcttttttgcacaacatgggggatcatgtaactcgccttgatcgttgggaaccggagctgaatgaagccataccaaacgacgagcgtgacaccacgatgcctgtagcaatggcaacaacgttgcgcaaactattaactggcgaactacttactctagcttcccggcaacaattaatagactggatggaggcggataaagttgcaggaccacttctgcgctcggcccttccggctggctggtttattgctgataaatctggagccggtgagcgtgggtctcgcggtatcattgcagcactggggccagatggtaagccctcccgtatcgtagttatctacacgacggggagtcaggcaactatggatgaacgaaatagacagatcgctgagataggtgcctcactgattaagcattggtaactgtcagaccaagtttactcatatatactttagattgatttaaaacttcatttttaatttaaaaggatctaggtgaagatcctttttgataatctcatgaccaaaatcccttaacgtgagttttcgttccactgagcgtcagaccccgtagaaaagatcaaaggatcttcttgagatcctttttttctgcgcgtaatctgctgcttgcaaacaaaaaaaccaccgctaccagcggtggtttgtttgccggatcaagagctaccaactctttttccgaaggtaactggcttcagcagagcgcagataccaaatactgttcttctagtgtagccgtagttaggccaccacttcaagaactctgtagcaccgcctacatacctcgctctgctaatcctgttaccagtggctgctgccagtggcgataagtcgtgtcttaccgggttggactcaagacgatagttaccggataaggcgcagcggtcgggctgaacggggggttcgtgcacacagcccagcttggagcgaacgacctacaccgaactgagatacctacagcgtgagctatgagaaagcgccacgcttcccgaagggagaaaggcggacaggtatccggtaagcggcagggtcggaacaggagagcgcacgagggagcttccagggggaaacgcctggtatctttatagtcctgtcgggtttcgccacctctgacttgagcgtcgatttttgtgatgctcgtcaggggggcggagcctatggaaaaacgccagcaacgcggcctttttacggttcctggccttttgctggccttttgctcacatgttctttcctgcgttatcccctgattctgtggataaccgtattaccgcctttgagtgagctgataccgctcgccgcagccgaacgaccgagcgcagcgagtcagtgagcgaggaagcggaagagcgcccaatacgcaaaccgcctctccccgcgcgttggccgattcattaatgcagctggcacgacaggtttcccgactggaaagcgggcagtgagcgcaacgcaattaatgtgagttagctcactcattaggcaccccaggctttacactttatgcttccggctcgtatgttgtgtggaattgtgagcggataacaatttcacacaggaaacagctatgaccatgattacgccagatttaattaaggccttaattaggctgcgcgctcgctcgctcactgaggccgcccgggcaaagcccgggcgtcgggcgacctttggtcgcccggcctcagtgagcgagcgagcgcgcagagagggagtggccaactccatcactaggggttccttgtagttaatgattaacccgccatgctacttatctaccagggtaatggggatcctctagaactatagctagtcgacattgattattgactagttattaatagtaatcaattacggggtcattagttcatagcccatatatggagttccgcgttacataacttacggtaaatggcccgcctggctgaccgcccaacgacccccgcccattgacgtcaataatgacgtatgttcccatagtaacgccaatagggactttccattgacgtcaatgggtggactatttacggtaaactgcccacttggcagtacatcaagtgtatcatatgccaagtacgccccctattgacgtcaatgacggtaaatggcccgcctggcattatgcccagtacatgaccttatgggactttcctacttggcagtacatctacgtattagtcatcgctattaccatggtcgaggtgagccccacgttctgcttcactctccccatctcccccccctccccacccccaattttgtatttatttattttttaattattttgtgcagcgatgggggcggggggggggggggggcgcgcgccaggcggggcggggcggggcgaggggcggggcggggcgaggcggagaggtgcggcggcagccaatcagagcggcgcgctccgaaagtttccttttatggcgaggcggcggcggcggcggccctataaaaagcgaagcgcgcggcgggcggggagtcgctgcgacgctgccttcgccccgtgccccgctccgccgccgcctcgcgccgcccgccccggctctgactgaccgcgttactcccacaggtgagcgggcgggacggcccttctcctccgggctgtaattagcgcttggtttaatgacggcttgtttcttttctgtggctgcgtgaaagccttgaggggctccgggagggccctttgtgcggggggagcggctcggggggtgcgtgcgtgtgtgtgtgcgtggggagcgccgcgtgcggctccgcgctgcccggcggctgtgagcgctgcgggcgcggcgcggggctttgtgcgctccgcagtgtgcgcgaggggagcgcggccgggggcggtgccccgcggtgcggggggggctgcgaggggaacaaaggctgcgtgcggggtgtgtgcgtgggggggtgagcagggggtgtgggcgcgtcggtcgggctgcaaccccccctgcacccccctccccgagttgctgagcacggcccggcttcgggtgcggggctccgtacggggcgtggcgcggggctcgccgtgccgggcggggggtggcggcaggtgggggtgccgggcggggcggggccgcctcgggccggggagggctcgggggaggggcgcggcggcccccggagcgccggcggctgtcgaggcgcggcgagccgcagccattgccttttatggtaatcgtgcgagagggcgcagggacttcctttgtcccaaatctgtgcggagccgaaatctgggaggcgccgccgcaccccctctagcgggcgcggggcgaagcggtgcggcgccggcaggaaggaaatgggcggggagggccttcgtgcgtcgccgcgccgccgtccccttctccctctccagcctcggggctgtccgcggggggacggctgccttcgggggggacggggcagggcggggttcggcttctggcgtgtgaccggcggctctagagcctctgctaaccatgttcatgccttcttctttttcctacagctcctgggcaacgtgctggttattgtgctgtctcatcattttggcaaagaattcatggagttcgggctgagctgggtctttctggtggccctgctgaagggagtccagtgcgaggtgcagctgctggaatccggacctggcctggtgaaaccatctgagacactgagtctgacttgtgctgtctccggcctgtctatcagctccgatttctcctgggcatggattaggcagacccccggcaaggccctggaatatgtggggtacatccgcgggaacaccggagatacatactataatcctagtctgaagtcaaggctgactatctcaaaggacaccagcaaaaaccaaatctacctgaatctgtctagtgtcaccgctggcgatgccgccgtgtactattgcgcaagggaccgggtgtgcgacgatgactacggatactattacaccgaggtgtgcttcggcctggattcttgggggcagggaatcgtggtcacagtgtcaagcggcggaggaggcagcggaggaggagggtccggaggcgggggatctgcagaactggtcatgacacagtccccactgagcctgtccgtcgctccaggacagactgcatctattagttgtcgatcctctcagtccctggactatgctaacggcaatacctacctgtcttggtttcaccagcgaccaggacagccacctcggagactgatctatcagatttccaacagagattctggagtgcccgacaggttctcaggcagcggagcaggaactgagtttaccctgcgaatcagtcggatggaatcagatgacgtggggatctactactgcggacaggggaccacattcccacggacatttggacagggcactaaggtggagatcaaaacctgtggaggaggaagcaagccaccaacctgccctccatgtacatctcccgaactgctgggcgggcctagcgtgttcctgtttccccctaagcctaaagatacactgatgattagtagaaccccagaggtcacatgcgtggtcgtggacgtgtcccaggaagatcctgacgtgaagttcaactggtacgtgaatggcgccgaggtgcaccatgctcagactaaaccacgcgaaacccagtataatagtacataccgagtcgtgtcagtcctgacagtgactcaccaggattggctgaacggcaaggagtatacctgcaaggtgtctaacaaggccctgcccgcccctatccagaaaacaattagcaaggacaaagggcagccacgggaaccccaggtgtacactctgccaccctcaagagaggaactgactaagaaccaggtcagcctgacctgtctggtgaaaggcttctaccccagcgatatcgtcgtggagtgggaaagttcaggccagcctgagaatacttacaagactacccctccagtgctggatagcgacgggtcctatttcctgtacagcaagctgacagtggacaaatcccgctggcagcagggaaacgtcttttcctgttctgtgatgcatgaggccctgcacaatgcttacacccagaagagtctgtcactgagccccggcaaatgag

SEQ ID NO: 6 - protein, 510 aa, synthetic construct
  REGION 1..510: note = Synthetic Construct
MEFGLSWVFLVALLKGVQCEVQLLESGPGLVKPSETLSLTCAVSGLSISSDFSWAWIRQTPGKALEYVGYIRGNTGDTYYNPSLKSRLTISKDTSKNQIYLNLSSVTAGDAAVYYCARDRVCDDDYGYYYTEVCFGLDSWGQGIVVTVSSGGGGSGGGGSGGGGSAELVMTQSPLSLSVAPGQTASISCRSSQSLDYANGNTYLSWFHQRPGQPPRRLIYQISNRDSGVPDRFSGSGAGTEFTLRISRMESDDVGIYYCGQGTTFPRTFGQGTKVEIKTCGGGSKPPTCPPCTSPELLGGPSVFLFPPKPKDTLMISRTPEVTCVVVDVSQEDPDVKFNWYVNGAEVHHAQTKPRETQYNSTYRVVSVLTVTHQDWLNGKEYTCKVSNKALPAPIQKTISKDKGQPREPQVYTLPPSREELTKNQVSLTCLVKGFYPSDIVVEWESSGQPENTYKTTPPVLDSDGSYFLYSKLTVDKSRWQQGNVFSCSVMHEALHNAYTQKSLSLSPGK

SEQ ID NO: 7 - DNA, 819 bp, synthetic construct
  misc_feature 1..819: note = engineered aducanumab scFv coding sequence
  source 1..819: mol_type = other DNA
atgtacaagatgcagctgctgagctgtatcgccctgaccctggtgctggtggccaactctcaggtgcagctggtggaatctggcggcggagtggtgcagcctggcagaagcctgagactgagctgtgccgccagcggcttcgccttcagcagctacggaatgcactgggtgcgccaggcccctggcaaaggactggaatgggtggccgtgatttggttcgacggcaccaagaagtactacaccgacagcgtgaagggccggttcaccatcagccgggacaacagcaagaacaccctgtacctgcagatgaataccctgcgggccgaggacaccgccgtgtactactgcgccagagacagaggcatcggcgccagacggggcccttactacatggacgtgtggggcaagggcaccaccgtgacagtgtctggcggaggcggaagtggcggagggggatcaggcgggggaggcagcgatattcagatgacccagagccccagcagcctgagcgcctctgtgggcgacagagtgaccatcacctgtcgggccagccagagcatcagctcctacctgaactggtatcagcagaagcccggcaaggcccccaagctgctgatctatgccgcctccagtctgcagagcggcgtgcccagcagattttctggcagcggctccggcaccgacttcaccctgacaatcagctccctgcagcccgaggacttcgccacctactactgccagcagagctacagcacccccctgacattcggcggaggcaccaaggtggaaatcaagcaccaccaccatcaccactgatga

SEQ ID NO: 8 - protein, 271 aa, synthetic construct
  REGION 1..271: note = Aducanumab scFv construct amino acid sequence
  SIGNAL 1..20: note = IL2 secretion signal
  REGION 21..143
  REGION 144..158: note = MISC_FEATURE - Gly-Ser Llinker
  REGION 159..265: note = MISC_FEATURE - Light Variable region
  REGION 266..271: note = MISC_FEATURE - 6xHistag (Explasy)
MYKMQLLSCIALTLVLVANSQVQLVESGGGVVQPGRSLRLSCAASGFAFSSYGMHWVRQAPGKGLEWVAVIWFDGTKKYYTDSVKGRFTISRDNSKNTLYLQMNTLRAEDTAVYYCARDRGIGARRGPYYMDVWGKGTTVTVSGGGGSGGGGSGGGGSDIQMTQSPSSLSASVGDRVTITCRASQSISSYLNWYQQKPGKAPKLLIYAASSLQSGVPSRFSGSGSGTDFTLTISSLQPEDFATYYCQQSYSTPLTFGGGTKVEIKHHHHHH

SEQ ID NO: 9 - DNA, 798 bp, synthetic construct
  misc_feature 1..798: note = Engineered crenezumab scFv construct
  source 1..798: mol_type = other DNA
atgtacaagatgcagctgctgagctgtatcgccctgaccctggtgctggtggccaactctgaagtgcagctggtggaaagcggcggaggcctggtgcagcctggcggatctctgagactgagctgtgccgccagcggcttcaccttcagcagctacggcatgagctgggtgcgccaggcccctggaaaaggcctggaactggtggcctccatcaacagcaatggcggcagcacctactaccccgacagcgtgaagggccggttcaccatctcccgggacaacgccaagaacagcctgtacctgcagatgaactccctgcgggccgaggacaccgccgtgtactattgtgccagcggcgactattggggccagggcacaaccgtgacagtgtctggcggaggcggatctgggggcggaggatcaggcgggggaggatctgatatcgtgatgacccagagccccctgagcctgcctgtgacacctggcgaacctgccagcatcagctgcagatccagccagagcctggtgtacagcaacggcgacacctacctgcactggtatctgcagaagcccggccagagccctcagctgctgatctacaaggtgtccaaccggttcagcggcgtgcccgacagattttctggcagcggctccggcaccgacttcaccctgaagatcagccgggtggaagccgaggacgtgggcgtgtactactgcagccagtccacccacgtgccctggacatttggacagggcaccaaggtggaaatcaagcaccaccaccatcaccactgatga

SEQ ID NO: 10 - protein, 264 aa, synthetic construct
  REGION 1..264: note = Engineered Crenezumab scFv amino acid sequence
  SIGNAL 1..20: note = IL-2 secretion signal
  REGION 21..131: note = MISC_FEATURE - Heavy variable region
  REGION 131..146: note = MISC_FEATURE - Gly-Ser Linker
  REGION 147..258: note = MISC_FEATURE - Light Variable Region
  REGION 259..264: note = MISC_FEATURE - 6xHis tag
MYKMQLLSCIALTLVLVANSEVQLVESGGGLVQPGGSLRLSCAASGFTFSSYGMSWVRQAPGKGLELVASINSNGGSTYYPDSVKGRFTISRDNAKNSLYLQMNSLRAEDTAVYYCASGDYWGQGTTVTVSGGGGSGGGGSGGGGSDIVMTQSPLSLPVTPGEPASISCRSSQSLVYSNGDTYLHWYLQKPGQSPQLLIYKVSNRFSGVPDRFSGSGSGTDFTLKISRVEAEDVGVYYCSQSTHVPWTFGQGTKVEIKHHHHHH

SEQ ID NO: 11 - DNA, 798 bp, synthetic construct
  misc_feature 1..798: note = engineered Solanezumab scFv construct nucleic acid sequence
  source 1..798: mol_type = other DNA
atgtacaagatgcagctgctgagctgtatcgccctgaccctggtgctggtggccaactctgaagtgcagctggtggaaagcggcggaggcctggtgcagcctggcggatctctgagactgagctgtgccgccagcggcttcaccttcagccggtacagcatgagctgggtgcgccaggcccctggcaaaggactggaactggtggcccagatcaacagcgtgggcaacagcacctactaccccgacaccgtgaagggccggttcaccatcagcagagacaacgccaagaacaccctgtacctgcagatgaacagcctgcgggccgaggacaccgccgtgtactattgtgccagcggcgactattggggccagggcacactcgtgacagtgtctggcggaggcggatctgggggcggaggatcaggcgggggaggatctgatgtcgtgatgacccagagccccctgagcctgcctgtgacactgggacagcctgccagcatcagctgcagaagcagccagagcctgatctacagcgacggcaacgcctacctgcactggtttctgcagaaacccggccagtcccccagactgctgatctataaggtgtccaaccggttcagcggcgtgcccgacagattttctggcagcggctccggcaccgacttcaccctgaagatcagccgggtggaagccgaggacgtgggcgtgtactactgcagccagtccacccacgtgccctggacatttggacagggcaccaaggtggaaatcaagcaccaccaccatcaccactgatga

SEQ ID NO: 12 - protein, 264 aa, synthetic construct
  REGION 1..264: note = engineered Solanezumab scFv construct amino acid sequence
  SIGNAL 1..20: note = IL2 secretion signal
  REGION 21..131: note = MISC_FEATURE - Heavy chain variable
  REGION 132..146
  REGION 147..258: note = MISC_FEATURE - Variable Light Region
  REGION 259..264: note = MISC_FEATURE - 6xHis tag
MYKMQLLSCIALTLVLVANSEVQLVESGGGLVQPGGSLRLSCAASGFTFSRYSMSWVRQAPGKGLELVAQINSVGNSTYYPDTVKGRFTISRDNAKNTLYLQMNSLRAEDTAVYYCASGDYWGQGTLVTVSGGGGSGGGGSGGGGSDVVMTQSPLSLPVTLGQPASISCRSSQSLIYSDGNAYLHWFLQKPGQSPRLLIYKVSNRFSGVPDRFSGSGSGTDFTLKISRVEAEDVGVYYCSQSTHVPWTFGQGTKVEIKHHHHHH

SEQ ID NO: 13 - DNA, 3165 bp, synthetic construct
  misc_feature 1..3165: note = AAV vector genome CB7.CI.aducanumabscFvRBG
  repeat_region 1..130: note = 5' AAV2-ITR
  repeat_region 198..579: note = CMV IE promoter
  regulatory 582..863: note = promoter - CB promoter; regulatory_class = promoter
  regulatory 836..838: regulatory_class = TATA_box
  misc_feature 958..1930: note = Intron - chicken beta actin promoter
  misc_feature 1958..2001
  misc_feature 2002..2370: note = aducanumab heavy variable region
  misc_feature 2371..2415: note = Gly-Ser Linker
  misc_feature 2416..2736: note = aducanumab light chain variable
  misc_feature 2737..2754: note = His Tag
  regulatory 2821..2947: note = polyA_signal - Rabbit globulin polya; regulatory_class = polyA_signal_sequence
  repeat_region 3036..3165: note = 3' ITR
  source 1..3165: mol_type = other DNA
ctgcgcgctcgctcgctcactgaggccgcccgggcaaagcccgggcgtcgggcgacctttggtcgcccggcctcagtgagcgagcgagcgcgcagagagggagtggccaactccatcactaggggttccttgtagttaatgattaacccgccatgctacttatctaccagggtaatggggatcctctagaactatagctagtcgacattgattattgactagttattaatagtaatcaattacggggtcattagttcatagcccatatatggagttccgcgttacataacttacggtaaatggcccgcctggctgaccgcccaacgacccccgcccattgacgtcaataatgacgtatgttcccatagtaacgccaatagggactttccattgacgtcaatgggtggactatttacggtaaactgcccacttggcagtacatcaagtgtatcatatgccaagtacgccccctattgacgtcaatgacggtaaatggcccgcctggcattatgcccagtacatgaccttatgggactttcctacttggcagtacatctacgtattagtcatcgctattaccatggtcgaggtgagccccacgttctgcttcactctccccatctcccccccctccccacccccaattttgtatttatttattttttaattattttgtgcagcgatgggggcggggggggggggggggcgcgcgccaggcggggcggggcggggcgaggggcggggcggggcgaggcggagaggtgcggcggcagccaatcagagcggcgcgctccgaaagtttccttttatggcgaggcggcggcggcggcggccctataaaaagcgaagcgcgcggcgggcggggagtcgctgcgacgctgccttcgccccgtgccccgctccgccgccgcctcgcgccgcccgccccggctctgactgaccgcgttactcccacaggtgagcgggcgggacggcccttctcctccgggctgtaattagcgcttggtttaatgacggcttgtttcttttctgtggctgcgtgaaagccttgaggggctccgggagggccctttgtgcggggggagcggctcggggggtgcgtgcgtgtgtgtgtgcgtggggagcgccgcgtgcggctccgcgctgcccggcggctgtgagcgctgcgggcgcggcgcggggctttgtgcgctccgcagtgtgcgcgaggggagcgcggccgggggcggtgccccgcggtgcggggggggctgcgaggggaacaaaggctgcgtgcggggtgtgtgcgtgggggggtgagcagggggtgtgggcgcgtcggtcgggctgcaaccccccctgcacccccctccccgagttgctgagcacggcccggcttcgggtgcggggctccgtacggggcgtggcgcggggctcgccgtgccgggcggggggtggcggcaggtgggggtgccgggcggggcggggccgcctcgggccggggagggctcgggggaggggcgcggcggcccccggagcgccggcggctgtcgaggcgcggcgagccgcagccattgccttttatggtaatcgtgcgagagggcgcagggacttcctttgtcccaaatctgtgcggagccgaaatctgggaggcgccgccgcaccccctctagcgggcgcggggcgaagcggtgcggcgccggcaggaaggaaatgggcggggagggccttcgtgcgtcgccgcgccgccgtccccttctccctctccagcctcggggctgtccgcggggggacggctgccttcgggggggacggggcagggcggggttcggcttctggcgtgtgaccggcggctctagagcctctgctaaccatgttcatgccttcttctttttcctacagctcctgggcaacgtgctggttattgtgctgtctcatcattttggcaaagaattcgccaccatgtacaagatgcagctgctgagctgtatcgccctgaccctggtgctggtggccaactctcaggtgcagctggtggaatctggcggcggagtggtgcagcctggcagaagcctgagactgagctgtgccgccagcggcttcgccttcagcagctacggaatgcactgggtgcgccaggcccctggcaaaggactggaatgggtggccgtgatttggttcgacggcaccaagaagtactacaccgacagcgtgaagggccggttcaccatcagccgggacaacagcaagaacaccctgtacctgcagatgaataccctgcgggccgaggacaccgccgtgtactactgcgccagagacagaggcatcggcgccagacggggcccttactacatggacgtgtggggcaagggcaccaccgtgacagtgtctggcggaggcggaagtggcggagggggatcaggcgggggaggcagcgatattcagatgacccagagccccagcagcctgagcgcctctgtgggcgacagagtgaccatcacctgtcgggccagccagagcatcagctcctacctgaactggtatcagcagaagcccggcaaggcccccaagctgctgatctatgccgcctccagtctgcagagcggcgtgcccagcagattttctggcagcggctccggcaccgacttcaccctgacaatcagctccctgcagcccgaggacttcgccacctactactgccagcagagctacagcacccccctgacattcggcggaggcaccaaggtggaaatcaagcaccaccaccatcaccactgatgaggtacctctagagtcgacccgggcggcctcgaggacggggtgaactacgcctgaggatccgatctttttccctctgccaaaaattatggggacatcatgaagccccttgagcatctgacttctggctaataaaggaaatttattttcattgcaatagtgtgttggaattttttgtgtctctcactcggaagcaattcgttgatctgaatttcgaccacccataatacccattaccctggtagataagtagcatggcgggttaatcattaactacaaggaacccctagtgatggagttggccactccctctctgcgcgctcgctcgctcactgaggccgggcgaccaaaggtcgcccgacgcccgggctttgcccgggcggcctcagtgagcgagcgagcgcgcag

SEQ ID NO: 14 - DNA, 3144 bp, synthetic construct
  misc_feature 1..3144: note = pAAV.CB7.CI.crenezumabScFv.RBG
  repeat_region 1..130: note = AAV2 - 5' ITR
  repeat_region 198..579: note = CMV IE promoter
  regulatory 582..863: note = promoter - CB promoter; regulatory_class = promoter
  regulatory 836..839: regulatory_class = TATA_box
  misc_feature 958..1930: note = Intron
  misc_feature 1942..2001: note = IL-2 secretion signal
  misc_feature 2001..2334: note = crenezumab heavy variable region
  misc_feature 2335..2379: note = Gly-Ser linker
  misc_feature 2380..2715: note = crenezumab varalbe region light
  misc_feature 2716..2733: note = His tag
  regulatory 2800..2926: note = polyA_signal - rabbit globin polyA; regulatory_class = polyA_signal_sequence
  repeat_region 3015..3144: note = AAV2 - 3' ITR
  source 1..3144: mol_type = other DNA
ctgcgcgctcgctcgctcactgaggccgcccgggcaaagcccgggcgtcgggcgacctttggtcgcccggcctcagtgagcgagcgagcgcgcagagagggagtggccaactccatcactaggggttccttgtagttaatgattaacccgccatgctacttatctaccagggtaatggggatcctctagaactatagctagtcgacattgattattgactagttattaatagtaatcaattacggggtcattagttcatagcccatatatggagttccgcgttacataacttacggtaaatggcccgcctggctgaccgcccaacgacccccgcccattgacgtcaataatgacgtatgttcccatagtaacgccaatagggactttccattgacgtcaatgggtggactatttacggtaaactgcccacttggcagtacatcaagtgtatcatatgccaagtacgccccctattgacgtcaatgacggtaaatggcccgcctggcattatgcccagtacatgaccttatgggactttcctacttggcagtacatctacgtattagtcatcgctattaccatggtcgaggtgagccccacgttctgcttcactctccccatctcccccccctccccacccccaattttgtatttatttattttttaattattttgtgcagcgatgggggcggggggggggggggggcgcgcgccaggcggggcggggcggggcgaggggcggggcggggcgaggcggagaggtgcggcggcagccaatcagagcggcgcgctccgaaagtttccttttatggcgaggcggcggcggcggcggccctataaaaagcgaagcgcgcggcgggcggggagtcgctgcgacgctgccttcgccccgtgccccgctccgccgccgcctcgcgccgcccgccccggctctgactgaccgcgttactcccacaggtgagcgggcgggacggcccttctcctccgggctgtaattagcgcttggtttaatgacggcttgtttcttttctgtggctgcgtgaaagccttgaggggctccgggagggccctttgtgcggggggagcggctcggggggtgcgtgcgtgtgtgtgtgcgtggggagcgccgcgtgcggctccgcgctgcccggcggctgtgagcgctgcgggcgcggcgcggggctttgtgcgctccgcagtgtgcgcgaggggagcgcggccgggggcggtgccccgcggtgcggggggggctgcgaggggaacaaaggctgcgtgcggggtgtgtgcgtgggggggtgagcagggggtgtgggcgcgtcggtcgggctgcaaccccccctgcacccccctccccgagttgctgagcacggcccggcttcgggtgcggggctccgtacggggcgtggcgcggggctcgccgtgccgggcggggggtggcggcaggtgggggtgccgggcggggcggggccgcctcgggccggggagggctcgggggaggggcgcggcggcccccggagcgccggcggctgtcgaggcgcggcgagccgcagccattgccttttatggtaatcgtgcgagagggcgcagggacttcctttgtcccaaatctgtgcggagccgaaatctgggaggcgccgccgcaccccctctagcgggcgcggggcgaagcggtgcggcgccggcaggaaggaaatgggcggggagggccttcgtgcgtcgccgcgccgccgtccccttctccctctccagcctcggggctgtccgcggggggacggctgccttcgggggggacggggcagggcggggttcggcttctggcgtgtgaccggcggctctagagcctctgctaaccatgttcatgccttcttctttttcctacagctcctgggcaacgtgctggttattgtgctgtctcatcattttggcaaagaattcgccaccatgtacaagatgcagctgctgagctgtatcgccctgaccctggtgctggtggccaactctgaagtgcagctggtggaaagcggcggaggcctggtgcagcctggcggatctctgagactgagctgtgccgccagcggcttcaccttcagcagctacggcatgagctgggtgcgccaggcccctggaaaaggcctggaactggtggcctccatcaacagcaatggcggcagcacctactaccccgacagcgtgaagggccggttcaccatctcccgggacaacgccaagaacagcctgtacctgcagatgaactccctgcgggccgaggacaccgccgtgtactattgtgccagcggcgactattggggccagggcacaaccgtgacagtgtctggcggaggcggatctgggggcggaggatcaggcgggggaggatctgatatcgtgatgacccagagccccctgagcctgcctgtgacacctggcgaacctgccagcatcagctgcagatccagccagagcctggtgtacagcaacggcgacacctacctgcactggtatctgcagaagcccggccagagccctcagctgctgatctacaaggtgtccaaccggttcagcggcgtgcccgacagattttctggcagcggctccggcaccgacttcaccctgaagatcagccgggtggaagccgaggacgtgggcgtgtactactgcagccagtccacccacgtgccctggacatttggacagggcaccaaggtggaaatcaagcaccaccaccatcaccactgatgaggtacctctagagtcgacccgggcggcctcgaggacggggtgaactacgcctgaggatccgatctttttccctctgccaaaaattatggggacatcatgaagccccttgagcatctgacttctggctaataaaggaaatttattttcattgcaatagtgtgttggaattttttgtgtctctcactcggaagcaattcgttgatctgaatttcgaccacccataatacccattaccctggtagataagtagcatggcgggttaatcattaactacaaggaacccctagtgatggagttggccactccctctctgcgcgctcgctcgctcactgaggccgggcgaccaaaggtcgcccgacgcccgggctttgcccgggcggcctcagtgagcgagcgagcgcgcag

SEQ ID NO: 15 - DNA, 3144 bp, synthetic construct
  misc_feature 1..3144: note = pAAV.CB7.CI.solanezumabscFv.RBG
  repeat_region 1..130: note = AAV2 - 5' ITR
  repeat_region 198..579: note = CMV IE promoter
  regulatory 582..863: note = promoter - CB promoter; regulatory_class = promoter
  regulatory 836..839: regulatory_class = TATA_box
  misc_feature 958..1930: note = Intron - chicken beta-actin intron
  misc_feature 1942..2001: note = IL-2 secretion signal
  misc_feature 2002..2334: note = solanezumab heavy variable region
  misc_feature 2335..2379: note = Gly-Ser Linker
  misc_feature 2380..2715: note = solanezumab light chain variable region
  regulatory 2800..2926: note = polyA_signal - rabbit globin polyA; regulatory_class = polyA_signal_sequence
  misc_feature 3015..3144: note = AAV2 - 3' ITR
  source 1..3144: mol_type = other DNA
ctgcgcgctcgctcgctcactgaggccgcccgggcaaagcccgggcgtcgggcgacctttggtcgcccggcctcagtgagcgagcgagcgcgcagagagggagtggccaactccatcactaggggttccttgtagttaatgattaacccgccatgctacttatctaccagggtaatggggatcctctagaactatagctagtcgacattgattattgactagttattaatagtaatcaattacggggtcattagttcatagcccatatatggagttccgcgttacataacttacggtaaatggcccgcctggctgaccgcccaacgacccccgcccattgacgtcaataatgacgtatgttcccatagtaacgccaatagggactttccattgacgtcaatgggtggactatttacggtaaactgcccacttggcagtacatcaagtgtatcatatgccaagtacgccccctattgacgtcaatgacggtaaatggcccgcctggcattatgcccagtacatgaccttatgggactttcctacttggcagtacatctacgtattagtcatcgctattaccatggtcgaggtgagccccacgttctgcttcactctccccatctcccccccctccccacccccaattttgtatttatttattttttaattattttgtgcagcgatgggggcggggggggggggggggcgcgcgccaggcggggcggggcggggcgaggggcggggcggggcgaggcggagaggtgcggcggcagccaatcagagcggcgcgctccgaaagtttccttttatggcgaggcggcggcggcggcggccctataaaaagcgaagcgcgcggcgggcggggagtcgctgcgacgctgccttcgccccgtgccccgctccgccgccgcctcgcgccgcccgccccggctctgactgaccgcgttactcccacaggtgagcgggcgggacggcccttctcctccgggctgtaattagcgcttggtttaatgacggcttgtttcttttctgtggctgcgtgaaagccttgaggggctccgggagggccctttgtgcggggggagcggctcggggggtgcgtgcgtgtgtgtgtgcgtggggagcgccgcgtgcggctccgcgctgcccggcggctgtgagcgctgcgggcgcggcgcggggctttgtgcgctccgcagtgtgcgcgaggggagcgcggccgggggcggtgccccgcggtgcggggggggctgcgaggggaacaaaggctgcgtgcggggtgtgtgcgtgggggggtgagcagggggtgtgggcgcgtcggtcgggctgcaaccccccctgcacccccctccccgagttgctgagcacggcccggcttcgggtgcggggctccgtacggggcgtggcgcggggctcgccgtgccgggcggggggtggcggcaggtgggggtgccgggcggggcggggccgcctcgggccggggagggctcgggggaggggcgcggcggcccccggagcgccggcggctgtcgaggcgcggcgagccgcagccattgccttttatggtaatcgtgcgagagggcgcagggacttcctttgtcccaaatctgtgcggagccgaaatctgggaggcgccgccgcaccccctctagcgggcgcggggcgaagcggtgcggcgccggcaggaaggaaatgggcggggagggccttcgtgcgtcgccgcgccgccgtccccttctccctctccagcctcggggctgtccgcggggggacggctgccttcgggggggacggggcagggcggggttcggcttctggcgtgtgaccggcggctctagagcctctgctaaccatgttcatgccttcttctttttcctacagctcctgggcaacgtgctggttattgtgctgtctcatcattttggcaaagaattcgccaccatgtacaagatgcagctgctgagctgtatcgccctgaccctggtgctggtggccaactctgaagtgcagctggtggaaagcggcggaggcctggtgcagcctggcggatctctgagactgagctgtgccgccagcggcttcaccttcagccggtacagcatgagctgggtgcgccaggcccctggcaaaggactggaactggtggcccagatcaacagcgtgggcaacagcacctactaccccgacaccgtgaagggccggttcaccatcagcagagacaacgccaagaacaccctgtacctgcagatgaacagcctgcgggccgaggacaccgccgtgtactattgtgccagcggcgactattggggccagggcacactcgtgacagtgtctggcggaggcggatctgggggcggaggatcaggcgggggaggatctgatgtcgtgatgacccagagccccctgagcctgcctgtgacactgggacagcctgccagcatcagctgcagaagcagccagagcctgatctacagcgacggcaacgcctacctgcactggtttctgcagaaacccggccagtcccccagactgctgatctataaggtgtccaaccggttcagcggcgtgcccgacagattttctggcagcggctccggcaccgacttcaccctgaagatcagccgggtggaagccgaggacgtgggcgtgtactactgcagccagtccacccacgtgccctggacatttggacagggcaccaaggtggaaatcaagcaccaccaccatcaccactgatgaggtacctctagagtcgacccgggcggcctcgaggacggggtgaactacgcctgaggatccgatctttttccctctgccaaaaattatggggacatcatgaagccccttgagcatctgacttctggctaataaaggaaatttattttcattgcaatagtgtgttggaattttttgtgtctctcactcggaagcaattcgttgatctgaatttcgaccacccataatacccattaccctggtagataagtagcatggcgggttaatcattaactacaaggaacccctagtgatggagttggccactccctctctgcgcgctcgctcgctcactgaggccgggcgaccaaaggtcgcccgacgcccgggctttgcccgggcggcctcagtgagcgagcgagcgcgcag